European Patent Application EP 4 357 365 A1, published April 24, 2024. Title: ANTIBODY TARGETING AXL PROTEIN AND ANTIGEN BINDING FRAGMENT THEREOF, AND PREPARATION METHOD THEREFOR AND APPLICATION THEREOF. Applicant: SHANGHAI SINOBAY BIOTECHNOLOGY CO., LTD. Application EP21945436.0. The sequence listing filed with the application follows.

SEQUENCE LISTING (32 sequences)

SEQ ID NO: 1 - protein, 124 aa, Artificial Sequence
  Heavy chain variable region (VH)
QVQLLESGGGVVQPGRSLRLSCAASGFTFSSYGMHWVRQAPGKGLEWVAVISYDGSNKYYADSVKGRFTISRDNSKNTLYLQMNSLRAEDTAVYYCAKDQVLAPVGGGLFDYWGQGTLVTVSAA

SEQ ID NO: 2 - protein, 107 aa, Artificial Sequence
  Light chain variable region (VL)
DIQLTQSPSSLSASVGDRVTITCRASQSISTYLNWYQQKPGKAPESLIFAASSLASGVPSRFSGSGSGTDFTLTISSLQPEDFATYYCQQSYSTPRTFGPGTKVEIK

SEQ ID NO: 3 - protein, 131 aa, Artificial Sequence
  Heavy chain variable region (VH)
QVQLVQSGAEVKKPGSSVKVSCKASGGTFSSYAISWVRQAPGQGLEWMGGIIPIFGTANYAQKFQGRVTITADESTSTAYMELSSLRSEDTAVYYCAKDIVSRVRGELVGGYYYFGLDVWGQGTTVTVSAA

SEQ ID NO: 4 - protein, 107 aa, Artificial Sequence
  Light chain variable region (VL)
NIQLTQSPSSLSASVGDRVTITCRASQTISSYLNWYQQKPGKAPKLLIYAASRLQSGVPSRFSGSGSGTDFTLTISSLQPEDFATYYCQQSYSTPRTFGQGTKVEIK

SEQ ID NO: 5 - protein, 122 aa, Artificial Sequence
  Heavy chain variable region (VH)
QVQLLESGGGVVQPGRSLRLSCAASGFTFSSYGMHWVRQAPGKGLEWVAVISYDGSNKYYADSVKGRFTISRDNSKNTLYLQMNSLRAEDTAVYYCAKYGSSGPYWYFDLWGQGTLVTVSAA

SEQ ID NO: 6 - protein, 107 aa, Artificial Sequence
  Light chain variable region (VL)
DIQLTQSPSSLSASVGDRVTITCRASQSISSYLNWYQQKPGKAPKLLIYAASSLQSGVPSRFSGSGSGTDFTLTISSLQPEDFATYYCQQSYSTPRTFGQGTKLEIR

SEQ ID NO: 7 - protein, 116 aa, Artificial Sequence
  Heavy chain variable region (VH)
EVQLVQSGAEVKKPGASVKVSCKASGYTFTSYYMHWVRQAPGQGLEWMGIINPSGGSTSYAQKFQGRVTMTRDTSTSTVYMELSSLRSEDSAVYYCARDWYFDVWGAGTTVTVSAA

SEQ ID NO: 8 - protein, 107 aa, Artificial Sequence
  Light chain variable region (VL)
NIQMTQSPSSVSASVGDRVTITCRASQGISSWLAWYQQKPGKAPKLLIYAASSLQSGVPSRFSGSGSGTDFTLTISSLQPEDFATYYCQQANSFPFTFGGGTKVEIK

SEQ ID NO: 9 - protein, 5 aa, Artificial Sequence
  Heavy chain variable region complementary determining region 1 (HCDR1)
SYGMH

SEQ ID NO: 10 - protein, 17 aa, Artificial Sequence
  Heavy chain variable region complementary determining region 2 (HCDR2)
VISYDGSNKYYADSVKG

SEQ ID NO: 11 - protein, 14 aa, Artificial Sequence
  Heavy chain variable region complementary determining region 3 (HCDR3)
DQVLAPVGGGLFDY

SEQ ID NO: 12 - protein, 11 aa, Artificial Sequence
  Light chain variable region complementary determining region 1 (LCDR1)
RASQSISTYLN

SEQ ID NO: 13 - protein, 7 aa, Artificial Sequence
  Light chain variable region complementary determining region 2 (LCDR2)
AASSLAS

SEQ ID NO: 14 - protein, 9 aa, Artificial Sequence
  Light chain variable region complementary determining region 3 (LCDR3)
QQSYSTPRT

SEQ ID NO: 15 - protein, 5 aa, Artificial Sequence
  Heavy chain variable region complementary determining region 1 (HCDR1)
SYAIS

SEQ ID NO: 16 - protein, 18 aa, Artificial Sequence
  Heavy chain variable region complementary determining region 2 (HCDR2)
GIIPIFGTANYAQKFQGR

SEQ ID NO: 17 - protein, 21 aa, Artificial Sequence
  Heavy chain variable region complementary determining region 3 (HCDR3)
DIVSRVRGELVGGYYYFGLDV

SEQ ID NO: 18 - protein, 9 aa, Artificial Sequence
  Light chain variable region complementary determining region 1 (LCDR1)
QQSYSTPRT

SEQ ID NO: 19 - protein, 7 aa, Artificial Sequence
  Light chain variable region complementary determining region 2 (LCDR2)
AASRLQS

SEQ ID NO: 20 - protein, 9 aa, Artificial Sequence
  Light chain variable region complementary determining region 3 (LCDR3)
QQSYSTPRT

SEQ ID NO: 21 - protein, 5 aa, Artificial Sequence
  Heavy chain variable region complementary determining region 1 (HCDR1)
SYGMH

SEQ ID NO: 22 - protein, 17 aa, Artificial Sequence
  Heavy chain variable region complementary determining region 2 (HCDR2)
VISYDGSNKYYADSVKG

SEQ ID NO: 23 - protein, 12 aa, Artificial Sequence
  Heavy chain variable region complementary determining region 3 (HCDR3)
YGSSGPYWYFDL

SEQ ID NO: 24 - protein, 11 aa, Artificial Sequence
  Light chain variable region complementary determining region 1 (LCDR1)
RASQSISSYLN

SEQ ID NO: 25 - protein, 7 aa, Artificial Sequence
  Light chain variable region complementary determining region 2 (LCDR2)
AASSLQS

SEQ ID NO: 26 - protein, 9 aa, Artificial Sequence
  Light chain variable region complementary determining region 3 (LCDR3)
QQSYSTPRT

SEQ ID NO: 27 - protein, 5 aa, Artificial Sequence
  Heavy chain variable region complementary determining region 1 (HCDR1)
SYYMH

SEQ ID NO: 28 - protein, 17 aa, Artificial Sequence
  Heavy chain variable region complementary determining region 2 (HCDR2)
IINPSGGSTSYAQKFQG

SEQ ID NO: 29 - protein, 6 aa, Artificial Sequence
  Heavy chain variable region complementary determining region 3 (HCDR3)
DWYFDV

SEQ ID NO: 30 - protein, 11 aa, Artificial Sequence
  Light chain variable region complementary determining region 1 (LCDR1)
RASQGISSWLA

SEQ ID NO: 31 - protein, 7 aa, Artificial Sequence
  Light chain variable region complementary determining region 2 (LCDR2)
AASSLQS

SEQ ID NO: 32 - protein, 8 aa, Artificial Sequence
  Light chain variable region complementary determining region 3 (LCDR3)
QQANSFPF